European Patent Specification EP 3 774 855 B1, published August 28, 2024. Title: An antimicrobial composition for selectively inhibiting growth of P. acnes bacteria. Applicant: Unilever PLC. The sequence listing filed with the application follows.

SEQUENCE LISTING (5 sequences)

SEQ ID NO: 1 - DNA, 20 bp, Staphylococcus capitis
agagtttgatcctggctcag

SEQ ID NO: 2 - DNA, 15 bp, Staphylococcus capitis
gggttgcgctcgttg

SEQ ID NO: 3 - DNA, 20 bp, Staphylococcus capitis
atccaagcttaaggaggtga

SEQ ID NO: 4 - DNA, 893 bp, Propionibacterium acnes
atgcgttatattccggcagcacatcattcagcaggtagcaatcatccggttaatcgtgttgttattcatgcaacctgtccggatgttggttttccgagcgcaagccgtaaaggtcgtgcagttagcaccgcaaactattttgcaagcccgagcagcggtggtagcgcacattatgtttgtgatattggtgaaaccgttcagtgtctgagcgaaggcaccattggttggcatgcaccgcctaatccgcatagcctgggtattgaaatttgtgcagatggtggtagccatgcaagctttcgtgttccgggtcatgcatatacccgtgaacagtggctggatccgcgtgtttggcctgcagttgaaaaagcagcaattctgtgtcgtcgtctgtgcgataaatacaatgttccgaaacgtaaactgagcgcagcagatctgaaagcaggtcgtcgtggtgtttgtggtcatgttgatgttaccgatgcatggcatcagagcgatcatgatgatccgggtccgtggtttccgtgggatcgttttatggcagttgttaatggtcataacgaaagcggtgaactgaccgttgcagatgttaaagcactgcatgatcagattaaacagctgagcgcacagctggcaggtagcgttaataaactgcatcatgatgttggtgttgttcaggttcagaatggtgatctgggtaaacgtgttgatgcactgagctgggttaaaaatccggttaccggtaaactgtggcgtaccaaagatgcactgtggtcagtttggtattatgttctggaatgtcgtagccgtattgatcgtctggaaagcgcagttaatggtctgaaaaaactcgagcaccaccaccaccaccactgagatccggctgctaa

SEQ ID NO: 5 - protein, 292 aa, Propionibacterium acnes
MRYIPAAHHSAGSNHPVNRVVIHATCPDVGFPSASRKGRAVSTANYFASPSSGGSAHYVCDIGETVQCLSEGTIGWHAPPNPHSLGIEICADGGSHASFRVPGHAYTREQWLDPRVWPAVEKAAILCRRLCDKYNVPKRKLSAADLKAGRRGVCGHVDVTDAWHQSDHDDPGPWFPWDRFMAVVNGHNESGELTVADVKALHDQIKQLSAQLAGSVNKLHHDVGVVQVQNGDLGKRVDALSWVKNPVTGKLWRTKDALWSVWYYVLECRSRIDRLESAVNGLKKLEHHHHHH